European Patent Application EP 4 421 167 A2, published August 28, 2024. Title: ENHANCED hAT FAMILY TRANSPOSON-MEDIATED GENE TRANSFER AND ASSOCIATED COMPOSITIONS, SYSTEMS, AND METHODS. Applicant: B-MOGEN BIOTECHNOLOGIES, INC. The sequence listing filed with the application follows.

SEQUENCE LISTING (203 sequences)

SEQ ID NO: 1 - protein, 636 aa, Tribolium castaneum
MMLNWLKSGKLESQSQEQSSCYLENSNCLPPTLDSTDIIGEENKAGTTSRKKRKYDEDYLNFGFTWTGDKDEPNGLCVICEQVVNNSSLNPAKLKRHLDTKHPTLKGKSEYFKRKCNELNQKKHTFERYVRDDNKNLLKASYLVSLRIAKQGEAYTIAEKLIKPCTKDLTTCVFGEKFASKVDLVPLSDTTISRRIEDMSYFCEAVLVNRLKNAKCGFTLQMDESTDVAGLAILLVFVRYIHESSFEEDMLFCKALPTQTTGEEIFNLLNAYFEKHSIPWNLCYHICTDGAKAMVGVIKGVIARIKKLVPDIKASHCCLHRHALAVKRIPNALHEVLNDAVKMINFIKSRPLNARVFALLCDDLGSLHKNLLLHTEVRWLSRGKVLTRFWELRDEIRIFFNEREFAGKLNDTSWLQNLAYIADIFSYLNEVNLSLQGPNSTIFKVNSRINSIKSKLKLWEECITKNNTECFANLNDFLETSNTALDPNLKSNILEHLNGLKNTFLEYFPPTCNNISWVENPFNECGNVDTLPIKEREQLIDIRTDTTLKSSFVPDGIGPFWIKLMDEFPEISKRAVKELMPFVTTYLCEKSFSVYVATKTKYRNRLDAEDDMRLQLTTIHPDIDNLCNNKQAQKSH

SEQ ID NO: 2 - DNA, 1911 bp, Tribolium castaneum
  source 1..1911: mol_type = other DNA
atgatgttgaattggctgaaaagtggaaagcttgaaagtcaatcacaggaacagagttcctgctaccttgagaactctaactgcctgccaccaacgctcgattctacagatattatcggtgaagagaacaaagctggtaccacctctcgcaagaagcggaaatatgacgaggactatctgaacttcggttttacatggactggcgacaaggatgagcccaacggactttgtgtgatttgcgagcaggtagtcaacaattcctcacttaacccggccaaactgaaacgccatttggacacaaagcatccgacgcttaaaggcaagagcgaatacttcaaaagaaaatgtaacgagctcaatcaaaagaagcatacttttgagcgatacgtaagggacgataacaagaacctcctgaaagcttcttatctcgtcagtttgagaatagctaaacagggcgaggcatataccatagcggagaagttgatcaagccttgcaccaaggatctgacaacttgcgtatttggagaaaaattcgcgagcaaagttgatctcgtccccctgtccgacacgactatttcaaggcgaatcgaagacatgagttacttctgtgaagccgtgctggtgaacaggttgaaaaatgctaaatgtgggtttacgctgcagatggacgagtcaacagatgttgccggtcttgcaatcctgcttgtgtttgttaggtacatacatgaaagctcttttgaggaggatatgttgttctgcaaagcacttcccactcagacgacaggggaggagattttcaatcttctcaatgcctatttcgaaaagcactccatcccatggaatctgtgttaccacatttgcacagacggtgccaaggcaatggtaggagttattaaaggagtcatagcgagaataaaaaaactcgtccctgatataaaagctagccactgttgcctgcatcgccacgctttggctgtaaagcgaataccgaatgcattgcacgaggtgctcaatgacgctgttaaaatgatcaacttcatcaagtctcggccgttgaatgcgcgcgtcttcgctttgctgtgtgacgatttggggagcctgcataaaaatcttcttcttcataccgaagtgaggtggctgtctagaggaaaggtgctgacccgattttgggaactgagagatgaaattagaattttcttcaacgaaagggaatttgccgggaaattgaacgacaccagttggttgcaaaatttggcatatatagctgacatattcagttatctgaatgaagttaatctttccctgcaagggccgaatagcacaatcttcaaggtaaatagccgcattaacagtattaaatcaaagttgaagttgtgggaagagtgtataacgaaaaataacactgagtgttttgcgaacctcaacgattttttggaaacttcaaacactgcgttggatccaaacctgaagtctaatattttggaacatctcaacggtcttaagaacacctttctggagtattttccacctacgtgtaataatatctcctgggtggagaatcctttcaatgaatgcggtaacgtcgatacactcccaataaaagagagggaacaattgattgacatacggactgatacgacattgaaatcttcattcgtgcctgatggtataggaccattctggatcaaactgatggacgaatttccagaaattagcaaacgagctgtcaaagagctcatgccatttgtaaccacttacctctgtgagaaatcattttccgtctatgtagccacaaaaacaaaatatcgaaatagacttgatgctgaagacgatatgcgactccaacttactactatccatccagacattgacaacctttgtaacaacaagcaggctcagaaatcccactga

SEQ ID NO: 3 - DNA, 458 bp, synthetic construct
  misc_feature 1..458: note = Description of Artificial Sequence: Synthetic polynucleotide
  source 1..458: mol_type = other DNA
cagtgttcttcaacctttgccatccggcggaaccctttgtcgagatatttttttttatggaacccttcatttagtaatacacccagatgagattttagggacagctgcgttgacttgttacgaacaaggtgagcccgtgctttggtctagccaagggcatggtaaagactatattcgcggcgttgtgacaatttaccgaacaactccgcggccgggaagccgatctcggcttgaacgaattgttaggtggcggtacttgggtcgatatcaaagtgcatcacttcttcccgtatgcccaactttgtatagagagccactgcgggatcgtcaccgtaatctgcttgcacgtagatcacataagcaccaagcgcgttggcctcatgcttgaggagattgatgagcgcggtggcaatgccctgcctccggtgctcgccggagactgcgagatcatagatata

SEQ ID NO: 4 - DNA, 361 bp, synthetic construct
  misc_feature 1..361: note = Description of Artificial Sequence: Synthetic polynucleotide
  source 1..361: mol_type = other DNA
gatatcaagcttatcgataccgtcgacctcgagatttctgaacgattctaggttaggatcaaacaaaatacaatttattttaaaactgtaagttaacttacctttgcttgtctaaaccaaaaacaacaacaaaactacgaccacaagtacagttacatatttttgaaaattaaggttaagtgcagtgtaagtcaactatgcgaatggataacatgtttcaacatgaaactccgattgacgcatgtgcattctgaagagcggcgcggccgacgtctctcgaattgaagcaatgactcgcggaaccccgaaagcctttgggtggaaccctagggttccgcggaacacaggttgaagaacactg

SEQ ID NO: 5 - DNA, 325 bp, synthetic construct
  misc_feature 1..325: note = Description of Artificial Sequence: Synthetic polynucleotide
  source 1..325: mol_type = other DNA
cctgcaggagtgttcttcaacctttgccatccggcggaaccctttgtcgagatatttttttttatggaacccttcatttagtaatacacccagatgagattttagggacagctgcgttgacttgttacgaacaaggtgagcccgtgctttggtaataaaaactctaaataagatttaaatttgcatttatttaaacaaactttaaacaaaaagataaatattccaaataaaataatatataaaataaaaaataaaaattaatgacttttttgcgcttgcttattattgcacaaattatcaatatcgggatggatcgttgtttttt

SEQ ID NO: 6 - DNA, 346 bp, synthetic construct
  misc_feature 1..346: note = Description of Artificial Sequence: Synthetic polynucleotide
  source 1..346: mol_type = other DNA
gagccaattcagcatcatatttctgaacgattctaggttaggatcaaacaaaatacaatttattttaaaactgtaagttaacttacctttgcttgtctaaacctaaaacaacaacaaaactacgaccacaagtacagttacatatttttgaaaattaaggttaagtgcagtgtaagtcaactatgcgaatggataacatgtttcaacatgaaactccgattgacgcatgtgcattctgaagagcggcgcggccgacgtctctcgaattgaagcaatgactcgcggaaccccgaaagcctttgggtggaaccctagggttccgcggaacacaggttgaagaacactg

SEQ ID NO: 7 - DNA, 7143 bp, synthetic construct
  misc_feature 1..7143: note = Description of Artificial Sequence: Synthetic polynucleotide
  source 1..7143: mol_type = other DNA
gacggatcgggagatctcccgatcccctatggtgcactctcagtacaatctgctctgatgccgcatagttaagccagtatctgctccctgcttgtgtgttggaggtcgctgagtagtgcgcgagcaaaatttaagctacaacaaggcaaggcttgaccgacaattgcatgaagaatctgcttagggttaggcgttttgcgctgcttcgcgatgtacgggccagatatacgcgttgacattgattattgactagttattaatagtaatcaattacggggtcattagttcatagcccatatatggagttccgcgttacataacttacggtaaatggcccgcctggctgaccgcccaacgacccccgcccattgacgtcaataatgacgtatgttcccatagtaacgccaatagggactttccattgacgtcaatgggtggagtatttacggtaaactgcccacttggcagtacatcaagtgtatcatatgccaagtacgccccctattgacgtcaatgacggtaaatggcccgcctggcattatgcccagtacatgaccttatgggactttcctacttggcagtacatctacgtattagtcatcgctattaccatggtgatgcggttttggcagtacatcaatgggcgtggatagcggtttgactcacggggatttccaagtctccaccccattgacgtcaatgggagtttgttttggcaccaaaatcaacgggactttccaaaatgtcgtaacaactccgccccattgacgcaaatgggcggtaggcgtgtacggtgggaggtctatataagcagagctctctggctaactagagaacccactgcttactggcttatcgaaattaatacgactcactatagggagacccaagctggctagttaagctatcaacaagtttgtacaaaaaagctgaacgagaaacgtaaaatgatataaatatcaatatattaaattagattttgcataaaaaacagactacataatactgtaaaacacaacatatccagtcactatggcggccgcattaggcaccccaggctttacactttatgcttccggctcgtataatgtgtggattttgagttaggatccggcgagattttcaggagctaaggaagctaaaatggagaaaaaaatcactggatataccaccgttgatatatcccaatggcatcgtaaagaacattttgaggcatttcagtcagttgctcaatgtacctataaccagaccgttcagctggatattacggcctttttaaagaccgtaaagaaaaataagcacaagttttatccggcctttattcacattcttgcccgcctgatgaatgctcatccggaattccgtatggcaatgaaagacggtgagctggtgatatgggatagtgttcacccttgttacaccgttttccatgagcaaactgaaacgttttcatcgctctggagtgaataccacgacgatttccggcagtttctacacatatattcgcaagatgtggcgtgttacggtgaaaacctggcctatttccctaaagggtttattgagaatatgtttttcgtctcagccaatccctgggtgagtttcaccagttttgatttaaacgtggccaatatggacaacttcttcgcccccgttttcaccatgggcaaatattatacgcaaggcgacaaggtgctgatgccgctggcgattcaggttcatcatgccgtctgtgatggcttccatgtcggcagaatgcttaatgaattacaacagtactgcgatgagtggcagggcggggcgtaaagatctggatccggcttactaaaagccagataacagtatgcgtatttgcgcgctgatttttgcggtataagaatatatactgatatgtatacccgaagtatgtcaaaaagaggtgtgctatgaagcagcgtattacagtgacagttgacagcgacagctatcagttgctcaaggcatatatgatgtcaatatctccggtctggtaagcacaaccatgcagaatgaagcccgtcgtctgcgtgccgaacgctggaaagcggaaaatcaggaagggatggctgaggtcgcccggtttattgaaatgaacggctcttttgctgacgagaacagggactggtgaaatgcagtttaaggtttacacctataaaagagagagccgttatcgtctgtttgtggatgtacagagtgatattattgacacgcccgggcgacggatggtgatccccctggccagtgcacgtctgctgtcagataaagtctcccgtgaactttacccggtggtgcatatcggggatgaaagctggcgcatgatgaccaccgatatggccagtgtgccggtctccgttatcggggaagaagtggctgatctcagccaccgcgaaaatgacatcaaaaacgccattaacctgatgttctggggaatataaatgtcaggctccgttatacacagccagtctgcaggtcgaccatagtgactggatatgttgtgttttacagtattatgtagtctgttttttatgcaaaatctaatttaatatattgatatttatatcattttacgtttctcgttcagctttcttgtacaaagtggttgatctagagggcccgcggttcgaaggtaagcctatccctaaccctctcctcggtctcgattctacgcgtaccggtcatcatcaccatcaccattgagtttaaacccgctgatcagcctcgactgtgccttctagttgccagccatctgttgtttgcccctcccccgtgccttccttgaccctggaaggtgccactcccactgtcctttcctaataaaatgaggaaattgcatcgcattgtctgagtaggtgtcattctattctggggggtggggtggggcaggacagcaagggggaggattgggaagacaatagcaggcatgctggggatgcggtgggctctatggcttctgaggcggaaagaaccagctggggctctagggggtatccccacgcgccctgtagcggcgcattaagcgcggcgggtgtggtggttacgcgcagcgtgaccgctacacttgccagcgccctagcgcccgctcctttcgctttcttcccttcctttctcgccacgttcgccggctttccccgtcaagctctaaatcgggggctccctttagggttccgatttagtgctttacggcacctcgaccccaaaaaacttgattagggtgatggttcacgtagtgggccatcgccctgatagacggtttttcgccctttgacgttggagtccacgttctttaatagtggactcttgttccaaactggaacaacactcaaccctatctcggtctattcttttgatttataagggattttgccgatttcggcctattggttaaaaaatgagctgatttaacaaaaatttaacgcgaattaattctgtggaatgtgtgtcagttagggtgtggaaagtccccaggctccccagcaggcagaagtatgcaaagcatgcatctcaattagtcagcaaccaggtgtggaaagtccccaggctccccagcaggcagaagtatgcaaagcatgcatctcaattagtcagcaaccatagtcccgcccctaactccgcccatcccgcccctaactccgcccagttccgcccattctccgccccatggctgactaattttttttatttatgcagaggccgaggccgcctctgcctctgagctattccagaagtagtgaggaggcttttttggaggcctaggcttttgcaaaaagctcccgggagcttgtatatccattttcggatctgatcaagagacaggatgaggatcgtttcgcatgattgaacaagatggattgcacgcaggttctccggccgcttgggtggagaggctattcggctatgactgggcacaacagacaatcggctgctctgatgccgccgtgttccggctgtcagcgcaggggcgcccggttctttttgtcaagaccgacctgtccggtgccctgaatgaactgcaggacgaggcagcgcggctatcgtggctggccacgacgggcgttccttgcgcagctgtgctcgacgttgtcactgaagcgggaagggactggctgctattgggcgaagtgccggggcaggatctcctgtcatctcaccttgctcctgccgagaaagtatccatcatggctgatgcaatgcggcggctgcatacgcttgatccggctacctgcccattcgaccaccaagcgaaacatcgcatcgagcgagcacgtactcggatggaagccggtcttgtcgatcaggatgatctggacgaagagcatcaggggctcgcgccagccgaactgttcgccaggctcaaggcgcgcatgcccgacggcgaggatctcgtcgtgacccatggcgatgcctgcttgccgaatatcatggtggaaaatggccgcttttctggattcatcgactgtggccggctgggtgtggcggaccgctatcaggacatagcgttggctacccgtgatattgctgaagagcttggcggcgaatgggctgaccgcttcctcgtgctttacggtatcgccgctcccgattcgcagcgcatcgccttctatcgccttcttgacgagttcttctgagcgggactctggggttcgcgaaatgaccgaccaagcgacgcccaacctgccatcacgagatttcgattccaccgccgccttctatgaaaggttgggcttcggaatcgttttccgggacgccggctggatgatcctccagcgcggggatctcatgctggagttcttcgcccaccccaacttgtttattgcagcttataatggttacaaataaagcaatagcatcacaaatttcacaaataaagcatttttttcactgcattctagttgtggtttgtccaaactcatcaatgtatcttatcatgtctgtataccgtcgacctctagctagagcttggcgtaatcatggtcatagctgtttcctgtgtgaaattgttatccgctcacaattccacacaacatacgagccggaagcataaagtgtaaagcctggggtgcctaatgagtgagctaactcacattaattgcgttgcgctcactgcccgctttccagtcgggaaacctgtcgtgccagctgcattaatgaatcggccaacgcgcggggagaggcggtttgcgtattgggcgctcttccgcttcctcgctcactgactcgctgcgctcggtcgttcggctgcggcgagcggtatcagctcactcaaaggcggtaatacggttatccacagaatcaggggataacgcaggaaagaacatgtgagcaaaaggccagcaaaaggccaggaaccgtaaaaaggccgcgttgctggcgtttttccataggctccgcccccctgacgagcatcacaaaaatcgacgctcaagtcagaggtggcgaaacccgacaggactataaagataccaggcgtttccccctggaagctccctcgtgcgctctcctgttccgaccctgccgcttaccggatacctgtccgcctttctcccttcgggaagcgtggcgctttctcatagctcacgctgtaggtatctcagttcggtgtaggtcgttcgctccaagctgggctgtgtgcacgaaccccccgttcagcccgaccgctgcgccttatccggtaactatcgtcttgagtccaacccggtaagacacgacttatcgccactggcagcagccactggtaacaggattagcagagcgaggtatgtaggcggtgctacagagttcttgaagtggtggcctaactacggctacactagaagaacagtatttggtatctgcgctctgctgaagccagttaccttcggaaaaagagttggtagctcttgatccggcaaacaaaccaccgctggtagcggtggtttttttgtttgcaagcagcagattacgcgcagaaaaaaaggatctcaagaagatcctttgatcttttctacggggtctgacgctcagtggaacgaaaactcacgttaagggattttggtcatgagattatcaaaaaggatcttcacctagatccttttaaattaaaaatgaagttttaaatcaatctaaagtatatatgagtaaacttggtctgacagttaccaatgcttaatcagtgaggcacctatctcagcgatctgtctatttcgttcatccatagttgcctgactccccgtcgtgtagataactacgatacgggagggcttaccatctggccccagtgctgcaatgataccgcgagacccacgctcaccggctccagatttatcagcaataaaccagccagccggaagggccgagcgcagaagtggtcctgcaactttatccgcctccatccagtctattaattgttgccgggaagctagagtaagtagttcgccagttaatagtttgcgcaacgttgttgccattgctacaggcatcgtggtgtcacgctcgtcgtttggtatggcttcattcagctccggttcccaacgatcaaggcgagttacatgatcccccatgttgtgcaaaaaagcggttagctccttcggtcctccgatcgttgtcagaagtaagttggccgcagtgttatcactcatggttatggcagcactgcataattctcttactgtcatgccatccgtaagatgcttttctgtgactggtgagtactcaaccaagtcattctgagaatagtgtatgcggcgaccgagttgctcttgcccggcgtcaatacgggataataccgcgccacatagcagaactttaaaagtgctcatcattggaaaacgttcttcggggcgaaaactctcaaggatcttaccgctgttgagatccagttcgatgtaacccactcgtgcacccaactgatcttcagcatcttttactttcaccagcgtttctgggtgagcaaaaacaggaaggcaaaatgccgcaaaaaagggaataagggcgacacggaaatgttgaatactcatactcttcctttttcaatattattgaagcatttatcagggttattgtctcatgagcggatacatatttgaatgtatttagaaaaataaacaaataggggttccgcgcacatttccccgaaaagtgccacctgacgtc

SEQ ID NO: 8 - DNA, 2844 bp, synthetic construct
  misc_feature 1..2844: note = Description of Artificial Sequence: Synthetic polynucleotide
  source 1..2844: mol_type = other DNA
atgctcgagatggatccctccgacgcttcgccggccgcgcaggtggatctacgcacgctcggctacagtcagcagcagcaagagaagatcaaaccgaaggtgcgttcgacagtggcgcagcaccacgaggcactggtgggccatgggtttacacacgcgcacatcgttgcgctcagccaacacccggcagcgttagggaccgtcgctgtcacgtatcagcacataatcacggcgttgccagaggcgacacacgaagacatcgttggcgtcggcaaacagtggtccggcgcacgcgccctggaggccttgttgactgatgctggtgagcttagaggacctcctttgcaacttgatacaggccagcttctgaaaatcgccaagaggggtggggtcaccgcggtcgaggccgtacacgcctggagaaatgcactgaccggggctcctcttaacctgaccccagaccaggtagtcgcaatcgcgtcaaacggagggggaaagcaagccctggaaaccgtgcaaaggttgttgccggtcctttgtcaagaccacggccttacaccggagcaagtcgtggccattgcatcccacgacggtggcaaacaggctcttgagacggttcagagacttctcccagttctctgtcaagcccacgggctgactcccgatcaagttgtagcgattgcgtcgcatgacggagggaaacaagcattggagactgtccaacggctccttcccgtgttgtgtcaagcccacggtttgacgcctgcacaagtggtcgccatcgcctccaatattggcggtaagcaggcgctggaaacagtacagcgcctgctgcctgtactgtgccaggatcatggactgacggccaagctggccgggggcgcccccgccgtgggcgggggccccaaggccgccgataaattcgccgccaccatgatgttgaattggctgaaaagtggaaagcttgaaagtcaatcacaggaacagagttcctgctaccttgagaactctaactgcctgccaccaacgctcgattctacagatattatcggtgaagagaacaaagctggtaccacctctcgcaagaagcggaaatatgacgaggactatctgaacttcggttttacatggactggcgacaaggatgagcccaacggactttgtgtgatttgcgagcaggtagtcaacaattcctcacttaacccggccaaactgaaacgccatttggacacaaagcatccgacgcttaaaggcaagagcgaatacttcaaaagaaaatgtaacgagctcaatcaaaagaagcatacttttgagcgatacgtaagggacgataacaagaacctcctgaaagcttcttatctcgtcagtttgagaatagctaaacagggcgaggcatataccatagcggagaagttgatcaagccttgcaccaaggatctgacaacttgcgtatttggagaaaaattcgcgagcaaagttgatctcgtccccctgtccgacacgactatttcaaggcgaatcgaagacatgagttacttctgtgaagccgtgctggtgaacaggttgaaaaatgctaaatgtgggtttacgctgcagatggacgagtcaacagatgttgccggtcttgcaatcctgcttgtgtttgttaggtacatacatgaaagctcttttgaggaggatatgttgttctgcaaagcacttcccactcagacgacaggggaggagattttcaatcttctcaatgcctatttcgaaaagcactccatcccatggaatctgtgttaccacatttgcacagacggtgccaaggcaatggtaggagttattaaaggagtcatagcgagaataaaaaaactcgtccctgatataaaagctagccactgttgcctgcatcgccacgctttggctgtaaagcgaataccgaatgcattgcacgaggtgctcaatgacgctgttaaaatgatcaacttcatcaagtctcggccgttgaatgcgcgcgtcttcgctttgctgtgtgacgatttggggagcctgcataaaaatcttcttcttcataccgaagtgaggtggctgtctagaggaaaggtgctgacccgattttgggaactgagagatgaaattagaattttcttcaacgaaagggaatttgccgggaaattgaacgacaccagttggttgcaaaatttggcatatatagctgacatattcagttatctgaatgaagttaatctttccctgcaagggccgaatagcacaatcttcaaggtaaatagccgcattaacagtattaaatcaaagttgaagttgtgggaagagtgtataacgaaaaataacactgagtgttttgcgaacctcaacgattttttggaaacttcaaacactgcgttggatccaaacctgaagtctaatattttggaacatctcaacggtcttaagaacacctttctggagtattttccacctacgtgtaataatatctcctgggtggagaatcctttcaatgaatgcggtaacgtcgatacactcccaataaaagagagggaacaattgattgacatacggactgatacgacattgaaatcttcattcgtgcctgatggtataggaccattctggatcaaactgatggacgaatttccagaaattagcaaacgagctgtcaaagagctcatgccatttgtaaccacttacctctgtgagaaatcattttccgtctatgtagccacaaaaacaaaatatcgaaatagacttgatgctgaagacgatatgcgactccaacttactactatccatccagacattgacaacctttgtaacaacaagcaggctcagaaatcccactga

SEQ ID NO: 9 - protein, 15 aa, synthetic construct
  REGION 1..15: note = Description of Artificial Sequence: Synthetic peptide
GGSGGSGGSGGSGTS

SEQ ID NO: 10 - DNA, 45 bp, synthetic construct
  misc_feature 1..45: note = Description of Artificial Sequence: Synthetic oligonucleotide
  source 1..45: mol_type = other DNA
ggaggtagtggcggtagtgggggctccggtgggagcggcacctca

SEQ ID NO: 11 - DNA, 863 bp, synthetic construct
  misc_feature 1..863: note = Description of Artificial Sequence: Synthetic polynucleotide
  source 1..863: mol_type = other DNA
atgctcgagatggatccctccgacgcttcgccggccgcgcaggtggatctacgcacgctcggctacagtcagcagcagcaagagaagatcaaaccgaaggtgcgttcgacagtggcgcagcaccacgaggcactggtgggccatgggtttacacacgcgcacatcgttgcgctcagccaacacccggcagcgttagggaccgtcgctgtcacgtatcagcacataatcacggcgttgccagaggcgacacacgaagacatcgttggcgtcggcaaacagtggtccggcgcacgcgccctggaggccttgttgactgatgctggtgagcttagaggacctcctttgcaacttgatacaggccagcttctgaaaatcgccaagaggggtggggtcaccgcggtcgaggccgtacacgcctggagaaatgcactgaccggggctcctcttaacctgaccccagaccaggtagtcgcaatcgcgtcaaacggagggggaaagcaagccctggaaaccgtgcaaaggttgttgccggtcctttgtcaagaccacggccttacaccggagcaagtcgtggccattgcatcccacgacggtggcaaacaggctcttgagacggttcagagacttctcccagttctctgtcaagcccacgggctgactcccgatcaagttgtagcgattgcgtcgcatgacggagggaaacaagcattggagactgtccaacggctccttcccgtgttgtgtcaagcccacggtttgacgcctgcacaagtggtcgccatcgcctccaatattggcggtaagcaggcgctggaaacagtacagcgcctgctgcctgtactgtgccaggatcatggactgac

SEQ ID NO: 12 - DNA, 70 bp, synthetic construct
  misc_feature 1..70: note = Description of Artificial Sequence: Synthetic oligonucleotide
  source 1..70: mol_type = other DNA
ggccaagctggccgggggcgcccccgccgtgggcgggggccccaaggccgccgataaattcgccgccacc

SEQ ID NO: 13 - protein, 636 aa, synthetic construct
  REGION 1..636: note = Description of Artificial Sequence: Synthetic polypeptide
MMLNWLKSGKLESQSQEQSSCYLENSNCLPPTLDSTDIIGEENKAGTTSRKKRKYDEDYLNFGFTWTGDKDEPNGLCVICEQVVNNSSLNPAKLKRHLDTKHPTLKGKSEYFKRKCNELNQKKHTFERYVRDDNKNLLKASYLVSLRIAKQGEAYTIAEKLIKPCTKDLTTCVFGEKFASKVDLVPLSATTISRRIEDMSYFCEAVLVNRLKNAKCGFTLQMDESTDVAGLAILLVFVRYIHESSFEEDMLFCKALPTQTTGEEIFNLLNAYFEKHSIPWNLCYHICTDGAKAMVGVIKGVIARIKKLVPDIKASHCCLHRHALAVKRIPNALHEVLNDAVKMINFIKSRPLNARVFALLCDDLGSLHKNLLLHTETRWLSRGKVLTRFWELRDEIRIFFNEREFAGKLNDTSWLQNLAYIADIFSYLNEVNLSLQGPNSTIFKVNSRINSIKSKLKLWEECITKNNTKCFANLNDFLETSNTALDPNLKSNILEHLNGLKNTFLEYFPPTCNNISWVENPFNECGNVDTLPIKEREQLIDIRTDTTLKSSFVPDGIGPFWIKLMDEFPEISERAVKLLMPFVTTYLCEKSFSVYVATKTKYRNRLDAEDDMRLQLTTIHPDIDNLCNNKQAQKSH

SEQ ID NO: 14 - DNA, 22 bp, synthetic construct
  misc_feature 1..22: note = Description of Artificial Sequence: Synthetic oligonucleotide
  source 1..22: mol_type = other DNA
gatttgcgaggaggtagtcaac

SEQ ID NO: 15 - DNA, 18 bp, synthetic construct
  misc_feature 1..18: note = Description of Artificial Sequence: Synthetic oligonucleotide
  source 1..18: mol_type = other DNA
acacaaagtccgttgggc

SEQ ID NO: 16 - DNA, 24 bp, synthetic construct
  misc_feature 1..24: note = Description of Artificial Sequence: Synthetic oligonucleotide
  source 1..24: mol_type = other DNA
cgcgtcttcgaattgctgtgtgac

SEQ ID NO: 17 - DNA, 18 bp, synthetic construct
  misc_feature 1..18: note = Description of Artificial Sequence: Synthetic oligonucleotide
  source 1..18: mol_type = other DNA
cgcattcaacggccgaga

SEQ ID NO: 18 - DNA, 26 bp, synthetic construct
  misc_feature 1..26: note = Description of Artificial Sequence: Synthetic oligonucleotide
  source 1..26: mol_type = other DNA
gcgcgtcttcagtttgctgtgtgacg

SEQ ID NO: 19 - DNA, 18 bp, synthetic construct
  misc_feature 1..18: note = Description of Artificial Sequence: Synthetic oligonucleotide
  source 1..18: mol_type = other DNA
gcattcaacggccgagac

SEQ ID NO: 20 - DNA, 26 bp, synthetic construct
  misc_feature 1..26: note = Description of Artificial Sequence: Synthetic oligonucleotide
  source 1..26: mol_type = other DNA
gcgcgtcttcaagttgctgtgtgacg

SEQ ID NO: 21 - DNA, 18 bp, synthetic construct
  misc_feature 1..18: note = Description of Artificial Sequence: Synthetic oligonucleotide
  source 1..18: mol_type = other DNA
gcattcaacggccgagac

SEQ ID NO: 22 - DNA, 33 bp, synthetic construct
  misc_feature 1..33: note = Description of Artificial Sequence: Synthetic oligonucleotide
  source 1..33: mol_type = other DNA
caaggtaaatgagcgcattaacagtattaaatc

SEQ ID NO: 23 - DNA, 18 bp, synthetic construct
  misc_feature 1..18: note = Description of Artificial Sequence: Synthetic oligonucleotide
  source 1..18: mol_type = other DNA
aagattgtgctattcggc

SEQ ID NO: 24 - DNA, 28 bp, synthetic construct
  misc_feature 1..28: note = Description of Artificial Sequence: Synthetic oligonucleotide
  source 1..28: mol_type = other DNA
cattaacagttttaaatcaaagttgaag

SEQ ID NO: 25 - DNA, 18 bp, synthetic construct
  misc_feature 1..18: note = Description of Artificial Sequence: Synthetic oligonucleotide
  source 1..18: mol_type = other DNA
cggctatttaccttgaag

SEQ ID NO: 26 - DNA, 23 bp, synthetic construct
  misc_feature 1..23: note = Description of Artificial Sequence: Synthetic oligonucleotide
  source 1..23: mol_type = other DNA
catcccatgggaactgtgttacc

SEQ ID NO: 27 - DNA, 19 bp, synthetic construct
  misc_feature 1..19: note = Description of Artificial Sequence: Synthetic oligonucleotide
  source 1..19: mol_type = other DNA
gagtgcttttcgaaatagg

SEQ ID NO: 28 - DNA, 26 bp, synthetic construct
  misc_feature 1..26: note = Description of Artificial Sequence: Synthetic oligonucleotide
  source 1..26: mol_type = other DNA
cggtcttgcacagctgcttgtgtttg

SEQ ID NO: 29 - DNA, 18 bp, synthetic construct
  misc_feature 1..18: note = Description of Artificial Sequence: Synthetic oligonucleotide
  source 1..18: mol_type = other DNA
gcaacatctgttgactcg

SEQ ID NO: 30 - DNA, 33 bp, synthetic construct
  misc_feature 1..33: note = Description of Artificial Sequence: Synthetic oligonucleotide
  source 1..33: mol_type = other DNA
gtattttccagatacgtgtaataatatctcctg

SEQ ID NO: 31 - DNA, 20 bp, synthetic construct
  misc_feature 1..20: note = Description of Artificial Sequence: Synthetic oligonucleotide
  source 1..20: mol_type = other DNA
tccagaaaggtgttcttaag

SEQ ID NO: 32 - DNA, 31 bp, synthetic construct
  misc_feature 1..31: note = Description of Artificial Sequence: Synthetic oligonucleotide
  source 1..31: mol_type = other DNA
gtattttccaaatacgtgtaataatatctcc

SEQ ID NO: 33 - DNA, 20 bp, synthetic construct
  misc_feature 1..20: note = Description of Artificial Sequence: Synthetic oligonucleotide
  source 1..20: mol_type = other DNA
tccagaaaggtgttcttaag

SEQ ID NO: 34 - DNA, 26 bp, synthetic construct
  misc_feature 1..26: note = Description of Artificial Sequence: Synthetic oligonucleotide
  source 1..26: mol_type = other DNA
ctcctgggtgcggaatcctttcaatg

SEQ ID NO: 35 - DNA, 20 bp, synthetic construct
  misc_feature 1..20: note = Description of Artificial Sequence: Synthetic oligonucleotide
  source 1..20: mol_type = other DNA
atattattacacgtaggtgg

SEQ ID NO: 36 - DNA, 21 bp, synthetic construct
  misc_feature 1..21: note = Description of Artificial Sequence: Synthetic oligonucleotide
  source 1..21: mol_type = other DNA
gaaattagcacacgagctgtc

SEQ ID NO: 37 - DNA, 18 bp, synthetic construct
  misc_feature 1..18: note = Description of Artificial Sequence: Synthetic oligonucleotide
  source 1..18: mol_type = other DNA
tggaaattcgtccatcag

SEQ ID NO: 38 - DNA, 23 bp, synthetic construct
  misc_feature 1..23: note = Description of Artificial Sequence: Synthetic oligonucleotide
  source 1..23: mol_type = other DNA
gcaggtagtcagcaattcctcac

SEQ ID NO: 39 - DNA, 19 bp, synthetic construct
  misc_feature 1..19: note = Description of Artificial Sequence: Synthetic oligonucleotide
  source 1..19: mol_type = other DNA
tcgcaaatcacacaaagtc

SEQ ID NO: 40 - DNA, 37 bp, synthetic construct
  misc_feature 1..37: note = Description of Artificial Sequence: Synthetic oligonucleotide
  source 1..37: mol_type = other DNA
taaaggcaaggacgaatacttcaaaagaaaatgtaac

SEQ ID NO: 41 - DNA, 37 bp, synthetic construct; identical to SEQ ID NO: 40
  misc_feature 1..37: note = Description of Artificial Sequence: Synthetic oligonucleotide
  source 1..37: mol_type = other DNA

SEQ ID NO: 42 - DNA, 23 bp, synthetic construct
  misc_feature 1..23: note = Description of Artificial Sequence: Synthetic oligonucleotide
  source 1..23: mol_type = other DNA
ggacgataacgagaacctcctga

SEQ ID NO: 43 - DNA, 23 bp, synthetic construct
  misc_feature 1..23: note = Description of Artificial Sequence: Synthetic oligonucleotide
  source 1..23: mol_type = other DNA
cttacgtatcgctcaaaagtatg

SEQ ID NO: 44 - DNA, 23 bp, synthetic construct
  misc_feature 1..23: note = Description of Artificial Sequence: Synthetic oligonucleotide
  source 1..23: mol_type = other DNA
acgccatttggcaacaaagcatc

SEQ ID NO: 45 - DNA, 18 bp, synthetic construct
  misc_feature 1..18: note = Description of Artificial Sequence: Synthetic oligonucleotide
  source 1..18: mol_type = other DNA
ttcagtttggccgggtta

SEQ ID NO: 46 - DNA, 26 bp, synthetic construct
  misc_feature 1..26: note = Description of Artificial Sequence: Synthetic oligonucleotide
  source 1..26: mol_type = other DNA
atacgtaagggcagataacaagaacc

SEQ ID NO: 47 - DNA, 18 bp, synthetic construct
  misc_feature 1..18: note = Description of Artificial Sequence: Synthetic oligonucleotide
  source 1..18: mol_type = other DNA
cgctcaaaagtatgcttc

SEQ ID NO: 48 - DNA, 25 bp, synthetic construct
  misc_feature 1..25: note = Description of Artificial Sequence: Synthetic oligonucleotide
  source 1..25: mol_type = other DNA
taccatagcggcgaagttgatcaag

SEQ ID NO: 49 - DNA, 18 bp, synthetic construct
  misc_feature 1..18: note = Description of Artificial Sequence: Synthetic oligonucleotide
  source 1..18: mol_type = other DNA
tatgcctcgccctgttta

SEQ ID NO: 50 - DNA, 24 bp, synthetic construct
  misc_feature 1..24: note = Description of Artificial Sequence: Synthetic oligonucleotide
  source 1..24: mol_type = other DNA
ccccctgtccgcaacgactatttc

SEQ ID NO: 51 - DNA, 18 bp, synthetic construct
  misc_feature 1..18: note = Description of Artificial Sequence: Synthetic oligonucleotide
  source 1..18: mol_type = other DNA
acgagatcaactttgctc

SEQ ID NO: 52 - DNA, 23 bp, synthetic construct
  misc_feature 1..23: note = Description of Artificial Sequence: Synthetic oligonucleotide
  source 1..23: mol_type = other DNA
cgagtcaacagcagttgccggtc

SEQ ID NO: 53 - DNA, 18 bp, synthetic construct
  misc_feature 1..18: note = Description of Artificial Sequence: Synthetic oligonucleotide
  source 1..18: mol_type = other DNA
tccatctgcagcgtaaac

SEQ ID NO: 54 - DNA, 23 bp, synthetic construct
  misc_feature 1..23: note = Description of Artificial Sequence: Synthetic oligonucleotide
  source 1..23: mol_type = other DNA
gtacatacatgcaagctcttttg

SEQ ID NO: 55 - DNA, 18 bp, synthetic construct
  misc_feature 1..18: note = Description of Artificial Sequence: Synthetic oligonucleotide
  source 1..18: mol_type = other DNA
ctaacaaacacaagcagg

SEQ ID NO: 56 - DNA, 24 bp, synthetic construct
  misc_feature 1..24: note = Description of Artificial Sequence: Synthetic oligonucleotide
  source 1..24: mol_type = other DNA
tcataccgaaacgaggtggctgtc

SEQ ID NO: 57 - DNA, 21 bp, synthetic construct
  misc_feature 1..21: note = Description of Artificial Sequence: Synthetic oligonucleotide
  source 1..21: mol_type = other DNA
agaagaagatttttatgcagg

SEQ ID NO: 58 - DNA, 24 bp, synthetic construct
  misc_feature 1..24: note = Description of Artificial Sequence: Synthetic oligonucleotide
  source 1..24: mol_type = other DNA
gatggacgagtggacagatgttgc

SEQ ID NO: 59 - DNA, 18 bp, synthetic construct
  misc_feature 1..18: note = Description of Artificial Sequence: Synthetic oligonucleotide
  source 1..18: mol_type = other DNA
tgcagcgtaaacccacat

SEQ ID NO: 60 - DNA, 23 bp, synthetic construct
  misc_feature 1..23: note = Description of Artificial Sequence: Synthetic oligonucleotide
  source 1..23: mol_type = other DNA
gggcgaggcatttaccatagcgg

SEQ ID NO: 61 - DNA, 31 bp, synthetic construct
  misc_feature 1..31: note = Description of Artificial Sequence: Synthetic oligonucleotide
  source 1..31: mol_type = other DNA
tgtttagctattctcaaactgacgagataag

SEQ ID NO: 62 - DNA, 26 bp, synthetic construct
  misc_feature 1..26: note = Description of Artificial Sequence: Synthetic oligonucleotide
  source 1..26: mol_type = other DNA
atacgtaagggcagataacaagaacc

SEQ ID NO: 63 - DNA, 18 bp, synthetic construct
  misc_feature 1..18: note = Description of Artificial Sequence: Synthetic oligonucleotide
  source 1..18: mol_type = other DNA
cgctcaaaagtatgcttc

SEQ ID NO: 64 - DNA, 25 bp, synthetic construct
  misc_feature 1..25: note = Description of Artificial Sequence: Synthetic oligonucleotide
  source 1..25: mol_type = other DNA
taccatagcggcgaagttgatcaag

SEQ ID NO: 65 - DNA, 18 bp, synthetic construct
  misc_feature 1..18: note = Description of Artificial Sequence: Synthetic oligonucleotide
  source 1..18: mol_type = other DNA
tatgcctcgccctgttta

SEQ ID NO: 66 - DNA, 24 bp, synthetic construct
  misc_feature 1..24: note = Description of Artificial Sequence: Synthetic oligonucleotide
  source 1..24: mol_type = other DNA
ccccctgtccgcaacgactatttc

SEQ ID NO: 67 - DNA, 18 bp, synthetic construct
  misc_feature 1..18: note = Description of Artificial Sequence: Synthetic oligonucleotide
  source 1..18: mol_type = other DNA
acgagatcaactttgctc

SEQ ID NO: 68 - DNA, 23 bp, synthetic construct
  misc_feature 1..23: note = Description of Artificial Sequence: Synthetic oligonucleotide
  source 1..23: mol_type = other DNA
cgagtcaacagcagttgccggtc

SEQ ID NO: 69 - DNA, 18 bp, synthetic construct
  misc_feature 1..18: note = Description of Artificial Sequence: Synthetic oligonucleotide
  source 1..18: mol_type = other DNA
tccatctgcagcgtaaac

SEQ ID NO: 70 - DNA, 23 bp, synthetic construct
  misc_feature 1..23: note = Description of Artificial Sequence: Synthetic oligonucleotide
  source 1..23: mol_type = other DNA
gtacatacatgcaagctcttttg

SEQ ID NO: 71 - DNA, 18 bp, synthetic construct
  misc_feature 1..18: note = Description of Artificial Sequence: Synthetic oligonucleotide
  source 1..18: mol_type = other DNA
ctaacaaacacaagcagg

SEQ ID NO: 72 - DNA, 24 bp, synthetic construct
  misc_feature 1..24: note = Description of Artificial Sequence: Synthetic oligonucleotide
  source 1..24: mol_type = other DNA
tcataccgaaacgaggtggctgtc

SEQ ID NO: 73 - DNA, 21 bp, synthetic construct
  misc_feature 1..21: note = Description of Artificial Sequence: Synthetic oligonucleotide
  source 1..21: mol_type = other DNA
agaagaagatttttatgcagg

SEQ ID NO: 74 - DNA, 24 bp, synthetic construct
  misc_feature 1..24: note = Description of Artificial Sequence: Synthetic oligonucleotide
  source 1..24: mol_type = other DNA
gatggacgagtggacagatgttgc

SEQ ID NO: 75 - DNA, 18 bp, synthetic construct
  misc_feature 1..18: note = Description of Artificial Sequence: Synthetic oligonucleotide
  source 1..18: mol_type = other DNA
tgcagcgtaaacccacat

SEQ ID NO: 76 - DNA, 23 bp, synthetic construct
  misc_feature 1..23: note = Description of Artificial Sequence: Synthetic oligonucleotide
  source 1..23: mol_type = other DNA
gggcgaggcatttaccatagcgg

SEQ ID NO: 77 - DNA, 31 bp, synthetic construct; identical to SEQ ID NO: 61
  misc_feature 1..31: note = Description of Artificial Sequence: Synthetic oligonucleotide
  source 1..31: mol_type = other DNA

SEQ ID NO: 78 - protein, 636 aa, synthetic construct
  REGION 1..636: note = Description of Artificial Sequence: Synthetic polypeptide
MMLNWLKSGKLESQSQEQSSCYLENSNCLPPTLDSTDIIGEENKAGTTSRKKRKYDEDYLNFGFTWTGDKDEPNGLCVICEQVVNNSSLNPAKLKRHLDTKHPTLKGKSEYFKRKCNELNQKKHTFERYVRDDNKNLLKASYLVSLRIAKQGEAYTIAEKLIKPCTKDLTTCVFGEKFASKVDLVPLSATTISRRIEDMSYFCEAVLVNRLKNAKCGFTLQMDESTDVAGLAILLVFVRYIHESSFEEDMLFCKALPTQTTGEEIFNLLNAYFEKHSIPWNLCYHICTDGAKAMVGVIKGVIARIKKLVPDIKASHCCLHRHALAVKRIPNALHEVLNDAVKMINFIKSRPLNARVFALLCDDLGSLHKNLLLHTETRWLSRGKVLTRFWELRDEIRIFFNEREFAGKLNDTSWLQNLAYIADIFSYLNEVNLSLQGPNSTIFKVNSRINSIKSKLKLWEECITKNNTKCFANLNDFLETSNTALDPNLKSNILEHLNGLKNTFLEYFPPTCNNISWVENPFNECGNVDTLPIKEREQLIDIRTDTTLKSSFVPDGIGPFWIKLMDEFPEISKRAVKELMPFVTTYLCEKSFSVYVATKTKYRNRLDAEDDMRLQLTTIHPDIDNLCNNKQAQKSH

SEQ ID NO: 79 - protein, 636 aa, synthetic construct
  REGION 1..636: note = Description of Artificial Sequence: Synthetic polypeptide
MMLNWLKSGKLESQSQEQSSCYLENSNCLPPTLDSTDIIGEENKAGTTSRKKRKYDEDYLNFGFTWTGDKDEPNGLCVICEQVVNNSSLNPAKLKRHLDTKHPTLKGKSEYFKRKCNELNQKKHTFERYVRDDNKNLLKASYLVSLRIAKQGEAYTIAEKLIKPCTKDLTTCVFGEKFASKVDLVPLSATTISRRIEDMSYFCEAVLVNRLKNAKCGFTLQMDESTDVAGLAILLVFVRYIHESSFEEDMLFCKALPTQTTGEEIFNLLNAYFEKHSIPWNLCYHICTDGAKAMVGVIKGVIARIKKLVPDIKASHCCLHRHALAVKRIPNALHEVLNDAVKMINFIKSRPLNARVFALLCDDLGSLHKNLLLHTETRWLSRGKVLTRFWELRDEIRIFFNEREFAGKLNDTSWLQNLAYIADIFSYLNEVNLSLQGPNSTIFKVNSRINSFKSKLKLWEECITKNNTKCFANLNDFLETSNTALDPNLKSNILEHLNGLKNTFLEYFPPTCNNISWVENPFNECGNVDTLPIKEREQLIDIRTDTTLKSSFVPDGIGPFWIKLMDEFPEISKRAVKELMPFVTTYLCEKSFSVYVATKTKYRNRLDAEDDMRLQLTTIHPDIDNLCNNKQAQKSH

SEQ ID NO: 80 - protein, 636 aa, synthetic construct
  REGION 1..636: note = Description of Artificial Sequence: Synthetic polypeptide
MMLNWLKSGKLESQSQEQSSCYLENSNCLPPTLDSTDIIGEENKAGTTSRKKRKYDEDYLNFGFTWTGDKDEPNGLCVICEQVVSNSSLNPAKLKRHLDTKHPTLKGKSEYFKRKCNELNQKKHTFERYVRDDNKNLLKASYLVSLRIAKQGEAYTIAEKLIKPCTKDLTTCVFGEKFASKVDLVPLSATTISRRIEDMSYFCEAVLVNRLKNAKCGFTLQMDESTDVAGLAILLVFVRYIHESSFEEDMLFCKALPTQTTGEEIFNLLNAYFEKHSIPWNLCYHICTDGAKAMVGVIKGVIARIKKLVPDIKASHCCLHRHALAVKRIPNALHEVLNDAVKMINFIKSRPLNARVFALLCDDLGSLHKNLLLHTETRWLSRGKVLTRFWELRDEIRIFFNEREFAGKLNDTSWLQNLAYIADIFSYLNEVNLSLQGPNSTIFKVNSRINSIKSKLKLWEECITKNNTKCFANLNDFLETSNTALDPNLKSNILEHLNGLKNTFLEYFPPTCNNISWVENPFNECGNVDTLPIKEREQLIDIRTDTTLKSSFVPDGIGPFWIKLMDEFPEISKRAVKELMPFVTTYLCEKSFSVYVATKTKYRNRLDAEDDMRLQLTTIHPDIDNLCNNKQAQKSH

SEQ ID NO: 81 - protein, 636 aa, synthetic construct
  REGION 1..636: note = Description of Artificial Sequence: Synthetic polypeptide
MMLNWLKSGKLESQSQEQSSCYLENSNCLPPTLDSTDIIGEENKAGTTSRKKRKYDEDYLNFGFTWTGDKDEPNGLCVICEQVVNNSSLNPAKLKRHLDTKHPTLKGKSEYFKRKCNELNQKKHTFERYVRDDNKNLLKASYLVSLRIAKQGEAYTIAEKLIKPCTKDLTTCVFGEKFASKVDLVPLSATTISRRIEDMSYFCEAVLVNRLKNAKCGFTLQMDESTDVAGLAILLVFVRYIHESSFEEDMLFCKALPTQTTGEEIFNLLNAYFEKHSIPWNLCYHICTDGAKAMVGVIKGVIARIKKLVPDIKASHCCLHRHALAVKRIPNALHEVLNDAVKMINFIKSRPLNARVFKLLCDDLGSLHKNLLLHTETRWLSRGKVLTRFWELRDEIRIFFNEREFAGKLNDTSWLQNLAYIADIFSYLNEVNLSLQGPNSTIFKVNSRINSIKSKLKLWEECITKNNTKCFANLNDFLETSNTALDPNLKSNILEHLNGLKNTFLEYFPPTCNNISWVENPFNECGNVDTLPIKEREQLIDIRTDTTLKSSFVPDGIGPFWIKLMDEFPEISKRAVKELMPFVTTYLCEKSFSVYVATKTKYRNRLDAEDDMRLQLTTIHPDIDNLCNNKQAQKSH

SEQ ID NO: 82 - skipped

SEQ ID NO: 83 - protein, 40 aa, synthetic construct
  REGION 1..40: note = Description of Artificial Sequence: Synthetic polypeptide
  VARIANT 1..40: note = This sequence may encompass 2-8 "Gly Gly Gly Gly Ser" repeating units
GGGGSGGGGSGGGGSGGGGSGGGGSGGGGSGGGGSGGGGS

SEQ ID NO: 84 - protein, 8 aa, synthetic construct
  REGION 1..8: note = Description of Artificial Sequence: Synthetic peptide
GGGGGGGG

SEQ ID NO: 85 - protein, 12 aa, synthetic construct
  REGION 1..12: note = Description of Artificial Sequence: Synthetic peptide
GSAGSAAGSGEF

SEQ ID NO: 86 - protein, 20 aa, synthetic construct
  REGION 1..20: note = Description of Artificial Sequence: Synthetic peptide
GGGGSGGGGSGGGGSGGGGS

SEQ ID NO: 87 - protein, 35 aa, synthetic construct
  REGION 1..35: note = Description of Artificial Sequence: Synthetic polypeptide
  VARIANT 1..35: note = This sequence may encompass 2-7 "Glu Ala Ala Ala Lys" repeating units
EAAAKEAAAKEAAAKEAAAKEAAAKEAAAKEAAAK

SEQ ID NO: 88 - protein, 6 aa, synthetic construct
  REGION 1..6: note = Description of Artificial Sequence: Synthetic peptide
GGGGSS

SEQ ID NO: 89 - protein, 7 aa, Tribolium castaneum
RHLDTKH

SEQ ID NO: 90 - protein, 6 aa, Tribolium castaneum
YVRDDN

SEQ ID NO: 91 - protein, 7 aa, Tribolium castaneum
EAYTIAE

SEQ ID NO: 92 - protein, 6 aa, Tribolium castaneum
GEKFAS

SEQ ID NO: 93 - protein, 5 aa, Tribolium castaneum
LSDTT

SEQ ID NO: 94 - protein, 5 aa, Tribolium castaneum
DESTD

SEQ ID NO: 95 - protein, 5 aa, Tribolium castaneum
RYIHE

SEQ ID NO: 96 - protein, 6 aa, Tribolium castaneum
TTGEEI

SEQ ID NO: 97 - protein, 7 aa, Tribolium castaneum
VRWLSRG

SEQ ID NO: 98 - protein, 5 aa, Tribolium castaneum
ECFAN

SEQ ID NO: 99 - protein, 5 aa, Tribolium castaneum
KEREQ

SEQ ID NO: 100 - protein, 4 aa, Tribolium castaneum
TKTK

SEQ ID NO: 101 - protein, 7 aa, Zea mays
NHLRTSH

SEQ ID NO: 102 - protein, 6 aa, Zea mays
YKYDEV

SEQ ID NO: 103 - protein, 7 aa, Zea mays
YPFNIVE

SEQ ID NO: 104 - protein, 6 aa, Zea mays
KSRVTA

SEQ ID NO: 105 - protein, 5 aa, Zea mays
LYLEE

SEQ ID NO: 106 - protein, 5 aa, Zea mays
DMWTS

SEQ ID NO: 107 - protein, 5 aa, Zea mays
HWIDD

SEQ ID NO: 108 - protein, 6 aa, Zea mays
HTGQRL

SEQ ID NO: 109 - protein, 7 aa, Zea mays
TRWNSTY

SEQ ID NO: 110 - protein, 5 aa, Zea mays
KYWKV

SEQ ID NO: 111 - protein, 5 aa, Zea mays
NDSMD

SEQ ID NO: 112 - protein, 4 aa, Zea mays
VVDP

SEQ ID NO: 113 - protein, 6 aa, Musca domestica
VSADCK

SEQ ID NO: 114 - protein, 7 aa, Musca domestica
RPFSAVS

SEQ ID NO: 115 - protein, 6 aa, Musca domestica
YGEHVN

SEQ ID NO: 116 - protein, 5 aa, Musca domestica
TSDAK

SEQ ID NO: 117 - protein, 5 aa, Musca domestica
DLWTD

SEQ ID NO: 118 - protein, 5 aa, Musca domestica
HYHEN

SEQ ID NO: 119 - protein, 6 aa, Musca domestica
STAENI

SEQ ID NO: 120 - protein, 7 aa, Musca domestica
TRWNSTY

SEQ ID NO: 121 - protein, 5 aa, Musca domestica
IIWEE

SEQ ID NO: 122 - protein, 5 aa, Musca domestica
HNSID

SEQ ID NO: 123 - protein, 4 aa, Musca domestica
IITE

SEQ ID NO: 124 - protein, 6 aa, Drosophila melanogaster
VSENDK

SEQ ID NO: 125 - protein, 7 aa, Drosophila melanogaster
RPFSAVT

SEQ ID NO: 126 - protein, 6 aa, Drosophila melanogaster
YGEQVD

SEQ ID NO: 127 - protein, 5 aa, Drosophila melanogaster
TSDAE

SEQ ID NO: 128 - protein, 5 aa, Drosophila melanogaster
DMWTD

SEQ ID NO: 129 - protein, 5 aa, Drosophila melanogaster
HYEKE

SEQ ID NO: 130 - protein, 6 aa, Drosophila melanogaster
STAENI

SEQ ID NO: 131 - protein, 7 aa, Drosophila melanogaster
TRWNSNY

SEQ ID NO: 132 - protein, 5 aa, Drosophila melanogaster
KIWMA

SEQ ID NO: 133 - protein, 5 aa, Drosophila melanogaster
PESLE

SEQ ID NO: 134 - protein, 4 aa, Drosophila melanogaster
IITE

SEQ ID NO: 135 - protein, 7 aa, Arabidopsis thaliana
RHMRSCE

SEQ ID NO: 136 - protein, 5 aa, Arabidopsis thaliana
KVDMM

SEQ ID NO: 137 - protein, 7 aa, Arabidopsis thaliana
LPYSFVE

SEQ ID NO: 138 - protein, 6 aa, Arabidopsis thaliana
WSRNTA

SEQ ID NO: 139 - protein, 5 aa, Arabidopsis thaliana
IYERE

SEQ ID NO: 140 - protein, 5 aa, Arabidopsis thaliana
DLWRA

SEQ ID NO: 141 - protein, 5 aa, Arabidopsis thaliana
HYVDV

SEQ ID NO: 142 - protein, 6 aa, Arabidopsis thaliana
HSGVAI

SEQ ID NO: 143 - protein, 7 aa, Arabidopsis thaliana
TRWNSTY

SEQ ID NO: 144 - protein, 5 aa, Arabidopsis thaliana
KYWED

SEQ ID NO: 145 - protein, 5 aa, Arabidopsis thaliana
QSSRK

SEQ ID NO: 146 - protein, 4 aa, Arabidopsis thaliana
VLNK

SEQ ID NO: 147 - protein, 7 aa, Antirrhinum majus
RHLTAKH

SEQ ID NO: 148 - protein, 6 aa, Antirrhinum majus
WRYDQN

SEQ ID NO: 149 - protein, 7 aa, Antirrhinum majus
LPFSFAQ

SEQ ID NO: 150 - protein, 6 aa, Antirrhinum majus
ISRATC

SEQ ID NO: 151 - protein, 5 aa, Antirrhinum majus
QYEKE

SEQ ID NO: 152 - protein, 5 aa, Antirrhinum majus
DLWQG

SEQ ID NO: 153 - protein, 5 aa, Antirrhinum majus
HWIDK

SEQ ID NO: 154 - protein, 6 aa, Antirrhinum majus
HNGDCI

SEQ ID NO: 155 - protein, 7 aa, Antirrhinum majus
HRWNATY

SEQ ID NO: 156 - protein, 5 aa, Antirrhinum majus
KYYKK

SEQ ID NO: 157 - protein, 5 aa, Antirrhinum majus
NASRG

SEQ ID NO: 158 - protein, 4 aa, Antirrhinum majus
VLTD

SEQ ID NO: 159 - protein, 7 aa, Anopheles gambiae
RHLNLVH

SEQ ID NO: 160 - protein, 6 aa, Anopheles gambiae
INSETK

SEQ ID NO: 161 - protein, 7 aa, Anopheles gambiae
LPFNLVE

SEQ ID NO: 162 - protein, 6 aa, Anopheles gambiae
PTRKSL

SEQ ID NO: 163 - protein, 5 aa, Anopheles gambiae
VYNQE

SEQ ID NO: 164 - protein, 5 aa, Anopheles gambiae
DGWTN

SEQ ID NO: 165 - protein, 5 aa, Anopheles gambiae
HYIDE

SEQ ID NO: 166 - protein, 6 aa, Anopheles gambiae
HSGRNI

SEQ ID NO: 167 - protein, 7 aa, Anopheles gambiae
TRWNSGY

SEQ ID NO: 168 - protein, 5 aa, Anopheles gambiae
KIYRS

SEQ ID NO: 169 - protein, 5 aa, Anopheles gambiae
KVSKD

SEQ ID NO: 170 - protein, 4 aa, Anopheles gambiae
IYSE

SEQ ID NO: 171 - protein, 7 aa, Tolypocladium inflatum
KHLRDIH

SEQ ID NO: 172 - protein, 6 aa, Tolypocladium inflatum
ILGRLK

SEQ ID NO: 173 - protein, 7 aa, Tolypocladium inflatum
LPFRLIE

SEQ ID NO: 174 - protein, 6 aa, Tolypocladium inflatum
YKDKVP

SEQ ID NO: 175 - protein, 5 aa, Tolypocladium inflatum
IYNGA

SEQ ID NO: 176 - protein, 5 aa, Tolypocladium inflatum
DGWTS

SEQ ID NO: 177 - protein, 5 aa, Tolypocladium inflatum
FFVDQ

SEQ ID NO: 178 - protein, 6 aa, Tolypocladium inflatum
HTGDNL

SEQ ID NO: 179 - protein, 7 aa, Tolypocladium inflatum
TRWNSRH

SEQ ID NO: 180 - protein, 5 aa, Tolypocladium inflatum
EYYDK

SEQ ID NO: 181 - protein, 5 aa, Tolypocladium inflatum
ASSRT

SEQ ID NO: 182 - protein, 4 aa, Tolypocladium inflatum
MVSP

SEQ ID NO: 183 - protein, 7 aa, Oryzias latipes
KHIERMH

SEQ ID NO: 184 - protein, 6 aa, Oryzias latipes
VKHVSP

SEQ ID NO: 185 - protein, 7 aa, Oryzias latipes
HPFSTVD

SEQ ID NO: 186 - protein, 6 aa, Oryzias latipes
ITRPTL

SEQ ID NO: 187 - protein, 5 aa, Oryzias latipes
AALIM

SEQ ID NO: 188 - protein, 5 aa, Oryzias latipes
DCWTA

SEQ ID NO: 189 - protein, 5 aa, Oryzias latipes
HWINP

SEQ ID NO: 190 - protein, 6 aa, Oryzias latipes
HTFEVL

SEQ ID NO: 191 - protein, 7 aa, Oryzias latipes
TRWNSTF

SEQ ID NO: 192 - protein, 5 aa, Oryzias latipes
RFKHM

SEQ ID NO: 193 - protein, 5 aa, Oryzias latipes
SSSDD

SEQ ID NO: 194 - protein, 4 aa, Oryzias latipes
LFSP

SEQ ID NO: 195 - protein, 41 aa, synthetic construct
  REGION 1..41: note = Description of Artificial Sequence: Synthetic polypeptide
DKDEPNGLCVICEQVVNNSSLNPAKLKRHLDTKHPTLKGKS

SEQ ID NO: 196 - protein, 41 aa, synthetic construct
  REGION 1..41: note = Description of Artificial Sequence: Synthetic polypeptide
FERYVRDDNKNLLKASYLVSLRIAKQGEAYTIAEKLIKPCT

SEQ ID NO: 197 - protein, 139 aa, synthetic construct
  REGION 1..139: note = Description of Artificial Sequence: Synthetic polypeptide
RRIEDMSYFCEAVLVNRLKNAKCGFTLQMDESTDVAGLAILLVFVRYIHESSFEEDMLFCKALPTQTTGEEIFNLLNAYFEKHSIPWNLCYHICTDGAKAMVGVIKGVIARIKKLVPDIKASHCCLHRHALAVKRIPNA

SEQ ID NO: 198 - protein, 63 aa, synthetic construct
  REGION 1..63: note = Description of Artificial Sequence: Synthetic polypeptide
AVKMINFIKSRPLNARVFALLCDDLGSLHKNLLLHTEVRWLSRGKVLTRFWELRDEIRIFFNE

SEQ ID NO: 199 - protein, 31 aa, synthetic construct
  REGION 1..31: note = Description of Artificial Sequence: Synthetic polypeptide
NLAYIADIFSYLNEVNLSLQGPNSTIFKVNS

SEQ ID NO: 200 - protein, 7 aa, synthetic construct
  REGION 1..7: note = Description of Artificial Sequence: Synthetic peptide
NSIKSKL

SEQ ID NO: 201 - protein, 7 aa, synthetic construct
  REGION 1..7: note = Description of Artificial Sequence: Synthetic peptide
ISWVENP

SEQ ID NO: 202 - protein, 62 aa, synthetic construct
  REGION 1..62: note = Description of Artificial Sequence: Synthetic polypeptide
IRTDTTLKSSFVPDGIGPFWIKLMDEFPEISKRAVKELMPFVTTYLCEKSFSVYVATKTKYR

SEQ ID NO: 203 - protein, 7 aa, synthetic construct
  REGION 1..7: note = Description of Artificial Sequence: Synthetic peptide
QLTTIHP